European Patent Specification EP 4 392 577 B1, published November 26, 2025. Title: IL-10 expressing cells for enhanced cancer immunotherapies. Applicant: ECOLE POLYTECHNIQUE FEDERALE DE LAUSANNE (EPFL). Application EP PCT/EP2022/073462, filed August 23, 2022. The sequence listing filed with the application follows.

SEQUENCE LISTING (7 sequences)

SEQ ID NO: 1 - protein, 160 aa, Homo sapiens
SPGQGTQSENSCTHFPGNLPNMLRDLRDAFSRVKTFFQMKDQLDNLLLKESLLEDFKGYLGCQALSEMIQFYLEEVMPQAENQDPDIKAHVNSLGENLKTLRLRLRRCHRFLPCENKSKAVEQVKNAFNKLQEKGIYKAMSEFDIFINYIEAYMTMKIRN

SEQ ID NO: 2 - protein, 252 aa, unidentified
  REGION 1..252: note = Artificial sequence
DYKDIVMTQSPSSLSASVGDRVTITCRASQDVNTAVAWYQQKPGKAPKLLIYSASFLYSGVPSRFSGSRSGTDFTLTISSLQPEDFATYYCQQHYTTPPTFGQGTKVELKRATPSHNSHQVPSAGGPTANSGEVKLVESGGGLVQPGGSLRLSCATSGFNIKDTYIHWVRQAPGKGLEWVARIYPTNGYTRYADSVKGRFTISADTSKNTAYLQMNSLRAEDTAVYYCSRWGGDGFYAMDYWGQGTTVTVSS

SEQ ID NO: 3 - protein, 245 aa, unidentified
  REGION 1..245: note = Artificial sequence
EVQLQQSGAELVRPGALVKLSCKTSGFNIKDYFLHWVRQRPDQGLEWIGWINPDNGNTVYDPKFQGTASLTADTSSNTVYLQLSGLTSEDTAVYFCTRRDYTYEKAALDYWGQGASVIVSSGGGGSGGGGSGGGGSDIQMSQSPASLSASVGETVTITCRASGNIYNYLAWYQQKQGKSPHLLVYDAKTLADGVPSRFSGSGSGTQYSLKISSLQTEDSGNYYCQHFWSLPFTFGSGTKLEIKRA

SEQ ID NO: 4 - protein, 238 aa, unidentified
  REGION 1..238: note = Artificial sequence
EVQVLESGGGLVQPGGSLRLSCAASGFTFSSYAMSWVRQAPGKGLEWVSAISGSGGSTNYADSVKGRFTISRDNSKNTLYLQMNSLRAEDTAVYYCAGSSGWSEYWGQGTLVTVSSGGGGSGGGGSGGGGSDIQMTQSPSSLSASVGDRVTITCRASQGIRNNLAWYQQKPGKAPKRLIYAASNLQSGVPSRFTGSGSGTEFTLIVSSLQPEDFATYYCLQHHSYPLTSGGGTKVEIK

SEQ ID NO: 5 - protein, 242 aa, unidentified
  REGION 1..242: note = Artificial sequence
DIQMTQTTSSLSASLGDRVTISCRASQDISKYLNWYQQKPDGTVKLLIYHTSRLHSGVPSRFSGSGSGTDYSLTISNLEQEDIATYFCQQGNTLPYTFGGGTKLEITGGGGSGGGGSGGGGSEVKLQESGPGLVAPSQSLSVTCTVSGVSLPDYGVSWIRQPPRKGLEWLGVIWGSETTYYNSALKSRLTIIKDNSKSQVFLKMNSLQTDDTAIYYCAKHYYYGGSYAMDYWGQGTSVTVSS

SEQ ID NO: 6 - protein, 72 aa, unidentified
  REGION 1..72: note = Artificial sequence
TTTKPVLRTPSPVHPTGTSQPQRPEDCRPRGSVKGTGLDFACDIYIWAPLAGICVALLLSLIITLICYHRSR

SEQ ID NO: 7 - protein, 113 aa, unidentified
  REGION 1..113: note = Artificial sequence
RAKFSRSAETAANLQDPNQLYNELNLGRREEYDVLEKKRARDPEMGGKQQRRRNPQEGVYNALQKDKMAEAYSEIGTKGERRRGKGHDGLYQGLSTATKDTYDALHMQTLAPR